European Patent Application EP 4 647 439 A1, published November 12, 2025. Title: NON-PATHOGENIC BACTERIA FOR DELIVERY OF PTD-FUSION PROTEINS. Applicant: Alma Mater Studiorum Università di Bologna. Application EP. The sequence listing filed with the application follows.

SEQUENCE LISTING (30 sequences)

SEQ ID NO: 1 - DNA, 40 bp, synthetic construct
  source 1..40: mol_type = other DNA
tattgagctctcaatgatgatgatgatgatggtcgacggc

SEQ ID NO: 2 - DNA, 116 bp, synthetic construct
  source 1..116: mol_type = other DNA
tattggtaccttatggctaaaaaaaagattatctcagctattttaatgtctacagtgatactttctgctgcagccccgttgtcaggtgtttacgctgacgcggcccagccggccag

SEQ ID NO: 3 - DNA, 37 bp, synthetic construct
  source 1..37: mol_type = other DNA
tattggtaccttatggctaaaaaaaagattatctcag

SEQ ID NO: 4 - DNA, 28 bp, synthetic construct
  source 1..28: mol_type = other DNA
tacagctccactctgtaaaagctgtcag

SEQ ID NO: 5 - DNA, 48 bp, synthetic construct
  source 1..48: mol_type = other DNA
ttttagccatatcttctcctaaatattcagtattaatataattatatc

SEQ ID NO: 6 - DNA, 35 bp, synthetic construct
  source 1..35: mol_type = other DNA
aggagaagatatggctaaaaaaaagattatctcag

SEQ ID NO: 7 - DNA, 54 bp, synthetic construct
  source 1..54: mol_type = other DNA
ttttggttcaattcagatcctcttctgagatgagtttttgttcgggccctcctc

SEQ ID NO: 8 - DNA, 33 bp, synthetic construct
  source 1..33: mol_type = other DNA
ggatctgaattgaaccaaaattagaaaaccaag

SEQ ID NO: 9 - DNA, 31 bp, synthetic construct
  source 1..31: mol_type = other DNA
ttttacagagtggagctgtaatataaaaacc

SEQ ID NO: 10 - DNA, 34 bp, synthetic construct
  source 1..34: mol_type = other DNA
gtacgaagaccacgctgtgagcaagggcgaggag

SEQ ID NO: 11 - DNA, 33 bp, synthetic construct
  source 1..33: mol_type = other DNA
gcgcgaagacgcagcgtaaacacctgacaacgg

SEQ ID NO: 12 - DNA, 34 bp, synthetic construct
  source 1..34: mol_type = other DNA
tattggtaccttatggagacagacacactcctgc

SEQ ID NO: 13 - DNA, 38 bp, synthetic construct
  source 1..38: mol_type = other DNA
tattgagctcctacttgtcatcgtcatccttgtagtcg

SEQ ID NO: 14 - DNA, 118 bp, synthetic construct
  source 1..118: mol_type = other DNA
tattggtaccttatggctaaaaaaaagattatctcagctattttaatgtctacagtgatactttctgctgcagccccgttgtcaggtgtttacgctatggagacagacacactcctgc

SEQ ID NO: 15 - DNA, 37 bp, synthetic construct; identical to SEQ ID NO: 3
  source 1..37: mol_type = other DNA

SEQ ID NO: 16 - DNA, 4139 bp, synthetic construct
  source 1..4139: mol_type = other DNA
ctagtcttataactatactgacaatagaaacattaacaaatctaaaacagtcttaattctatcttgagaaagtattggtaataatattattgtcgataacgcgagcataataaacggctctgattaaattctgaagtttgttagatacaatgatttcgttcgaaggaactacaaaataaattataaggaggcactcaccatgggtactgcaggcatgcggtaccttatggctaaaaaaaagattatctcagctattttaatgtctacagtgatactttctgctgcagccccgttgtcaggtgtttacgctgacgcggcccagccggccaggcgcgcgcgccgtacgaagcttgcggcctacgccagaaaggccgccaggcaggccagggcaccggtcgccactgtgagcaagggcgaggagctgttcaccggggtggtgcccatcctggtcgagctggacggcgacgtaaacggccacaagttcagcgtgtccggcgagggcgagggcgatgccacctacggcaagctgaccctgaagttcatctgcaccaccggcaagctgcccgtgccctggcccaccctcgtgaccaccctgacctacggcgtgcagtgcttcagccgctaccccgaccacatgaagcagcacgacttcttcaagtccgccatgcccgaaggctacgtccaggagcgcaccatcttcttcaaggacgacggcaactacaagacccgcgccgaggtgaagttcgagggcgacaccctggtgaaccgcatcgagctgaagggcatcgacttcaaggaggacggcaacatcctggggcacaagctggagtacaactacaacagccacaacgtctatatcatggccgacaagcagaagaacggcatcaaggtgaacttcaagatccgccacaacatcgaggacggcagcgtgcagctcgccgaccactaccagcagaacacccccatcggcgacggccccgtgctgctgcccgacaaccactacctgagcacccagtccgccctgagcaaagaccccaacgagaagcgcgatcacatggtcctgctggagttcgtgaccgccgccgggatcactctcggcatggacgagctgtacaagtccggactcagatctcgaggagggcccgaacaaaaactcatctcagaagaggatctgaatagcgccgtcgaccatcatcatcatcatcattgagagctcaagctttctttgaaccaaaattagaaaaccaaggcttgaaacgttcaattgaaatggcaattaaacaaattacagcacgtgttgctttgattgatagccaaaaagcagcagttgataaagcaattactgatattgctgaaaaattgtaatttataaataaaaatcaccttttagaggtggtttttttatttataaattattcgtttgatttcgctttcgatagaacaatcaaatcgtttctgagacgttttagcgtttatttcgtttagttatcggcataatcgttaaaacaggcgttatcgtagcgtaaaagcccttgagcgtagcgtgctttgcagcgaagatgttgtctgttagattatgaaagccgatgactgaatgaaataataagcgcagcgtccttctatttcggttggaggaggctcaagggagtttgagggaatgaaattccctcatgggtttgattttaaaaattgcttgcaattttgccgagcggtagcgctggaaaatttttgaaaaaaatttggaatttggaaaaaaatggggggaaaggaagcgaattttgcttccgtactacgaccccccattaagtgccgagtgccaatttttgtgccaaaaacgctctatcccaactggctcaagggtttgaggggtttttcaatcgccaacgaatcgccaacgttttcgccaacgttttttataaatctatatttaagtagctttattgttgtttttatgattacaaagtgatacactaattttataaaattatttgattggagttttttaaatggtgatttcagaatcgaaaaaaagagttatgatttctctgacaaaagagcaagataaaaaattaacagatatggcgaaacaaaaaggtttttcaaaatctgcggttgcggcgttagctatagaagaatatgcaagaaaggaatcagaacaaaaaaaataagcgaaagctcgcgtttttagaaggatacgagttttcgctacttgtttttgataaggtaatatatcatggctattaaaaatactaaagctagaaattttggatttttattatatcctgactcaattcctaatgattggaaagaaaaattagagagtttgggcgtatctatggctgtcagtcctttacacgatatggacgaaaaaaaagataaagatacatggaatagtagtgatgttatacgaaatggaaagcactataaaaaaccacactatcacgttatatatattgcacgaaatcctgtaacaatagaaagcgttaggaacaagattaagcgaaaattggggaatagttcagttgctcatgttgagatacttgattatatcaaaggttcatatgaatatttgactcatgaatcaaaggacgctattgctaagaataaacatatatacgacaaaaaagatattttgaacattaatgattttgatattgaccgctatataacacttgatgaaagccaaaaaagagaattgaagaatttacttttagatatagtggatgactataatttggtaaatacaaaagatttaatggcttttattcgccttaggggagcggagtttggaattttaaatacgaatgatgtaaaagatattgtttcaacaaactctagcgcctttagattatggtttgagggcaattatcagtgtggatatagagcaagttatgcaaaggttcttgatgctgaaacgggggaaataaaatgacaaacaaagaaaaagagttatttgctgaaaatgaggaattaaaaaaagaaattaaggacttaaaagagcgtattgaaagatacagagaaatggaagttgaattaagtacaacaatagatttattgagaggagggattattgaataaataaaagcccccctgacgaaagtcgacggcaatagttacccttattatcaagataagaaagaaaaggatttttcgctacgctcaaatcctttaaaaaaacacaaaagaccacattttttaatgtggtctttattcttcaactaaagcacccattagttcaacaaacgaaaattggataaagtgggatatttttaaaatatatatttatgttacagtaatattgacttttaaaaaaggattgattctaatgaagaaagcagacaagtaagcctcctaaattcactttagataaaaatttaggaggcatatcaaatgaactttaataaaattgatttagacaattggaagagaaaagagatatttaatcattatttgaaccaacaaacgacttttagtataaccacagaaattgatattagtgttttataccgaaacataaaacaagaaggatataaattttaccctgcatttattttcttagtgacaagggtgataaactcaaatacagcttttagaactggttacaatagcgacggagagttaggttattgggataagttagagccactttatacaatttttgatggtgtatctaaaacattctctggtatttggactcctgtaaagaatgacttcaaagagttttatgatttatacctttctgatgtagagaaatataatggttcggggaaattgtttcccaaaacacctatacctgaaaatgctttttctctttctattattccttggacttcatttactgggtttaacttaaatatcaataataatagtaattaccttctacccattattacagcaggaaaattcattaataaaggtaattcaatatatttaccgctatctttacaggtacatcattctgtttgtgatggttatcatgcaggattgtttatgaactctattcaggaattgtcagataggcctaatgactggcttttataatatgagataatgccgactgtactttttacagtcggttttctaatgtcactaacctgccccgttagttgaagaaggtttttatattacagctccaagat

SEQ ID NO: 17 - protein, 327 aa, synthetic construct
MAKKKIISAILMSTVILSAAAPLSGVYADAAQPARRARRTKLAAYARKAARQARAPVATVSKGEELFTGVVPILVELDGDVNGHKFSVSGEGEGDATYGKLTLKFICTTGKLPVPWPTLVTTLTYGVQCFSRYPDHMKQHDFFKSAMPEGYVQERTIFFKDDGNYKTRAEVKFEGDTLVNRIELKGIDFKEDGNILGHKLEYNYNSHNVYIMADKQKNGIKVNFKIRHNIEDGSVQLADHYQQNTPIGDGPVLLPDNHYLSTQSALSKDPNEKRDHMVLLEFVTAAGITLGMDELYKSGLRSRGGPEQKLISEEDLNSAVDHHHHHH

SEQ ID NO: 18 - DNA, 3987 bp, synthetic construct
  source 1..3987: mol_type = other DNA
ctctgtaaaagctgtcagtagacagtttttttaataagttaaagaaaagatgtaatttttctttgtactcgaaattttctattcaatttgatataattatattaatactgaatatttaggagaagatatggctaaaaaaaagattatctcagctattttaatgtctacagtgatactttctgctgcagccccgttgtcaggtgtttacgctgacgcggcccagccggccaggcgcgcgcgccgtacgaagcttgcggcctacgccagaaaggccgccaggcaggccagggcaccggtcgccactgtgagcaagggcgaggagctgttcaccggggtggtgcccatcctggtcgagctggacggcgacgtaaacggccacaagttcagcgtgtccggcgagggcgagggcgatgccacctacggcaagctgaccctgaagttcatctgcaccaccggcaagctgcccgtgccctggcccaccctcgtgaccaccctgacctacggcgtgcagtgcttcagccgctaccccgaccacatgaagcagcacgacttcttcaagtccgccatgcccgaaggctacgtccaggagcgcaccatcttcttcaaggacgacggcaactacaagacccgcgccgaggtgaagttcgagggcgacaccctggtgaaccgcatcgagctgaagggcatcgacttcaaggaggacggcaacatcctggggcacaagctggagtacaactacaacagccacaacgtctatatcatggccgacaagcagaagaacggcatcaaggtgaacttcaagatccgccacaacatcgaggacggcagcgtgcagctcgccgaccactaccagcagaacacccccatcggcgacggccccgtgctgctgcccgacaaccactacctgagcacccagtccgccctgagcaaagaccccaacgagaagcgcgatcacatggtcctgctggagttcgtgaccgccgccgggatcactctcggcatggacgagctgtacaagtccggactcagatctcgaggagggcccgaacaaaaactcatctcagaagaggatctgaattgaaccaaaattagaaaaccaaggcttgaaacgttcaattgaaatggcaattaaacaaattacagcacgtgttgctttgattgatagccaaaaagcagcagttgataaagcaattactgatattgctgaaaaattgtaatttataaataaaaatcaccttttagaggtggtttttttatttataaattattcgtttgatttcgctttcgatagaacaatcaaatcgtttctgagacgttttagcgtttatttcgtttagttatcggcataatcgttaaaacaggcgttatcgtagcgtaaaagcccttgagcgtagcgtgctttgcagcgaagatgttgtctgttagattatgaaagccgatgactgaatgaaataataagcgcagcgtccttctatttcggttggaggaggctcaagggagtttgagggaatgaaattccctcatgggtttgattttaaaaattgcttgcaattttgccgagcggtagcgctggaaaatttttgaaaaaaatttggaatttggaaaaaaatggggggaaaggaagcgaattttgcttccgtactacgaccccccattaagtgccgagtgccaatttttgtgccaaaaacgctctatcccaactggctcaagggtttgaggggtttttcaatcgccaacgaatcgccaacgttttcgccaacgttttttataaatctatatttaagtagctttattgttgtttttatgattacaaagtgatacactaattttataaaattatttgattggagttttttaaatggtgatttcagaatcgaaaaaaagagttatgatttctctgacaaaagagcaagataaaaaattaacagatatggcgaaacaaaaaggtttttcaaaatctgcggttgcggcgttagctatagaagaatatgcaagaaaggaatcagaacaaaaaaaataagcgaaagctcgcgtttttagaaggatacgagttttcgctacttgtttttgataaggtaatatatcatggctattaaaaatactaaagctagaaattttggatttttattatatcctgactcaattcctaatgattggaaagaaaaattagagagtttgggcgtatctatggctgtcagtcctttacacgatatggacgaaaaaaaagataaagatacatggaatagtagtgatgttatacgaaatggaaagcactataaaaaaccacactatcacgttatatatattgcacgaaatcctgtaacaatagaaagcgttaggaacaagattaagcgaaaattggggaatagttcagttgctcatgttgagatacttgattatatcaaaggttcatatgaatatttgactcatgaatcaaaggacgctattgctaagaataaacatatatacgacaaaaaagatattttgaacattaatgattttgatattgaccgctatataacacttgatgaaagccaaaaaagagaattgaagaatttacttttagatatagtggatgactataatttggtaaatacaaaagatttaatggcttttattcgccttaggggagcggagtttggaattttaaatacgaatgatgtaaaagatattgtttcaacaaactctagcgcctttagattatggtttgagggcaattatcagtgtggatatagagcaagttatgcaaaggttcttgatgctgaaacgggggaaataaaatgacaaacaaagaaaaagagttatttgctgaaaatgaggaattaaaaaaagaaattaaggacttaaaagagcgtattgaaagatacagagaaatggaagttgaattaagtacaacaatagatttattgagaggagggattattgaataaataaaagcccccctgacgaaagtcgacggcaatagttacccttattatcaagataagaaagaaaaggatttttcgctacgctcaaatcctttaaaaaaacacaaaagaccacattttttaatgtggtctttattcttcaactaaagcacccattagttcaacaaacgaaaattggataaagtgggatatttttaaaatatatatttatgttacagtaatattgacttttaaaaaaggattgattctaatgaagaaagcagacaagtaagcctcctaaattcactttagataaaaatttaggaggcatatcaaatgaactttaataaaattgatttagacaattggaagagaaaagagatatttaatcattatttgaaccaacaaacgacttttagtataaccacagaaattgatattagtgttttataccgaaacataaaacaagaaggatataaattttaccctgcatttattttcttagtgacaagggtgataaactcaaatacagcttttagaactggttacaatagcgacggagagttaggttattgggataagttagagccactttatacaatttttgatggtgtatctaaaacattctctggtatttggactcctgtaaagaatgacttcaaagagttttatgatttatacctttctgatgtagagaaatataatggttcggggaaattgtttcccaaaacacctatacctgaaaatgctttttctctttctattattccttggacttcatttactgggtttaacttaaatatcaataataatagtaattaccttctacccattattacagcaggaaaattcattaataaaggtaattcaatatatttaccgctatctttacaggtacatcattctgtttgtgatggttatcatgcaggattgtttatgaactctattcaggaattgtcagataggcctaatgactggcttttataatatgagataatgccgactgtactttttacagtcggttttctaatgtcactaacctgccccgttagttgaagaaggtttttatattacagctcca

SEQ ID NO: 19 - protein, 317 aa, synthetic construct
MAKKKIISAILMSTVILSAAAPLSGVYADAAQPARRARRTKLAAYARKAARQARAPVATVSKGEELFTGVVPILVELDGDVNGHKFSVSGEGEGDATYGKLTLKFICTTGKLPVPWPTLVTTLTYGVQCFSRYPDHMKQHDFFKSAMPEGYVQERTIFFKDDGNYKTRAEVKFEGDTLVNRIELKGIDFKEDGNILGHKLEYNYNSHNVYIMADKQKNGIKVNFKIRHNIEDGSVQLADHYQQNTPIGDGPVLLPDNHYLSTQSALSKDPNEKRDHMVLLEFVTAAGITLGMDELYKSGLRSRGGPEQKLISEEDLN

SEQ ID NO: 20 - DNA, 3894 bp, synthetic construct
  source 1..3894: mol_type = other DNA
ctctgtaaaagctgtcagtagacagtttttttaataagttaaagaaaagatgtaatttttctttgtactcgaaattttctattcaatttgatataattatattaatactgaatatttaggagaagatatggctaaaaaaaagattatctcagctattttaatgtctacagtgatactttctgctgcagccccgttgtcaggtgtttacgctgtgagcaagggcgaggagctgttcaccggggtggtgcccatcctggtcgagctggacggcgacgtaaacggccacaagttcagcgtgtccggcgagggcgagggcgatgccacctacggcaagctgaccctgaagttcatctgcaccaccggcaagctgcccgtgccctggcccaccctcgtgaccaccctgacctacggcgtgcagtgcttcagccgctaccccgaccacatgaagcagcacgacttcttcaagtccgccatgcccgaaggctacgtccaggagcgcaccatcttcttcaaggacgacggcaactacaagacccgcgccgaggtgaagttcgagggcgacaccctggtgaaccgcatcgagctgaagggcatcgacttcaaggaggacggcaacatcctggggcacaagctggagtacaactacaacagccacaacgtctatatcatggccgacaagcagaagaacggcatcaaggtgaacttcaagatccgccacaacatcgaggacggcagcgtgcagctcgccgaccactaccagcagaacacccccatcggcgacggccccgtgctgctgcccgacaaccactacctgagcacccagtccgccctgagcaaagaccccaacgagaagcgcgatcacatggtcctgctggagttcgtgaccgccgccgggatcactctcggcatggacgagctgtacaagtccggactcagatctcgaggagggcccgaacaaaaactcatctcagaagaggatctgaattgaaccaaaattagaaaaccaaggcttgaaacgttcaattgaaatggcaattaaacaaattacagcacgtgttgctttgattgatagccaaaaagcagcagttgataaagcaattactgatattgctgaaaaattgtaatttataaataaaaatcaccttttagaggtggtttttttatttataaattattcgtttgatttcgctttcgatagaacaatcaaatcgtttctgagacgttttagcgtttatttcgtttagttatcggcataatcgttaaaacaggcgttatcgtagcgtaaaagcccttgagcgtagcgtgctttgcagcgaagatgttgtctgttagattatgaaagccgatgactgaatgaaataataagcgcagcgtccttctatttcggttggaggaggctcaagggagtttgagggaatgaaattccctcatgggtttgattttaaaaattgcttgcaattttgccgagcggtagcgctggaaaatttttgaaaaaaatttggaatttggaaaaaaatggggggaaaggaagcgaattttgcttccgtactacgaccccccattaagtgccgagtgccaatttttgtgccaaaaacgctctatcccaactggctcaagggtttgaggggtttttcaatcgccaacgaatcgccaacgttttcgccaacgttttttataaatctatatttaagtagctttattgttgtttttatgattacaaagtgatacactaattttataaaattatttgattggagttttttaaatggtgatttcagaatcgaaaaaaagagttatgatttctctgacaaaagagcaagataaaaaattaacagatatggcgaaacaaaaaggtttttcaaaatctgcggttgcggcgttagctatagaagaatatgcaagaaaggaatcagaacaaaaaaaataagcgaaagctcgcgtttttagaaggatacgagttttcgctacttgtttttgataaggtaatatatcatggctattaaaaatactaaagctagaaattttggatttttattatatcctgactcaattcctaatgattggaaagaaaaattagagagtttgggcgtatctatggctgtcagtcctttacacgatatggacgaaaaaaaagataaagatacatggaatagtagtgatgttatacgaaatggaaagcactataaaaaaccacactatcacgttatatatattgcacgaaatcctgtaacaatagaaagcgttaggaacaagattaagcgaaaattggggaatagttcagttgctcatgttgagatacttgattatatcaaaggttcatatgaatatttgactcatgaatcaaaggacgctattgctaagaataaacatatatacgacaaaaaagatattttgaacattaatgattttgatattgaccgctatataacacttgatgaaagccaaaaaagagaattgaagaatttacttttagatatagtggatgactataatttggtaaatacaaaagatttaatggcttttattcgccttaggggagcggagtttggaattttaaatacgaatgatgtaaaagatattgtttcaacaaactctagcgcctttagattatggtttgagggcaattatcagtgtggatatagagcaagttatgcaaaggttcttgatgctgaaacgggggaaataaaatgacaaacaaagaaaaagagttatttgctgaaaatgaggaattaaaaaaagaaattaaggacttaaaagagcgtattgaaagatacagagaaatggaagttgaattaagtacaacaatagatttattgagaggagggattattgaataaataaaagcccccctgacgaaagtcgacggcaatagttacccttattatcaagataagaaagaaaaggatttttcgctacgctcaaatcctttaaaaaaacacaaaagaccacattttttaatgtggtctttattcttcaactaaagcacccattagttcaacaaacgaaaattggataaagtgggatatttttaaaatatatatttatgttacagtaatattgacttttaaaaaaggattgattctaatgaagaaagcagacaagtaagcctcctaaattcactttagataaaaatttaggaggcatatcaaatgaactttaataaaattgatttagacaattggaagagaaaagagatatttaatcattatttgaaccaacaaacgacttttagtataaccacagaaattgatattagtgttttataccgaaacataaaacaagaaggatataaattttaccctgcatttattttcttagtgacaagggtgataaactcaaatacagcttttagaactggttacaatagcgacggagagttaggttattgggataagttagagccactttatacaatttttgatggtgtatctaaaacattctctggtatttggactcctgtaaagaatgacttcaaagagttttatgatttatacctttctgatgtagagaaatataatggttcggggaaattgtttcccaaaacacctatacctgaaaatgctttttctctttctattattccttggacttcatttactgggtttaacttaaatatcaataataatagtaattaccttctacccattattacagcaggaaaattcattaataaaggtaattcaatatatttaccgctatctttacaggtacatcattctgtttgtgatggttatcatgcaggattgtttatgaactctattcaggaattgtcagataggcctaatgactggcttttataatatgagataatgccgactgtactttttacagtcggttttctaatgtcactaacctgccccgttagttgaagaaggtttttatattacagctcca

SEQ ID NO: 21 - protein, 286 aa, synthetic construct
MAKKKIISAILMSTVILSAAAPLSGVYAVSKGEELFTGVVPILVELDGDVNGHKFSVSGEGEGDATYGKLTLKFICTTGKLPVPWPTLVTTLTYGVQCFSRYPDHMKQHDFFKSAMPEGYVQERTIFFKDDGNYKTRAEVKFEGDTLVNRIELKGIDFKEDGNILGHKLEYNYNSHNVYIMADKQKNGIKVNFKIRHNIEDGSVQLADHYQQNTPIGDGPVLLPDNHYLSTQSALSKDPNEKRDHMVLLEFVTAAGITLGMDELYKSGLRSRGGPEQKLISEEDLN

SEQ ID NO: 22 - DNA, 6266 bp, synthetic construct
  source 1..6266: mol_type = other DNA
agatctagtcttataactatactgacaatagaaacattaacaaatctaaaacagtcttaattctatcttgagaaagtattggtaataatattattgtcgataacgcgagcataataaacggctctgattaaattctgaagtttgttagatacaatgatttcgttcgaaggaactacaaaataaattataaggaggcactcaccatgggtactgcaggcatgcggtaccttatggagacagacacactcctgctatgggtactgctgctctgggttccaggttccactggtgacgcggcccagccggccaggcgcgcgcgccgtacgaagcttgcggcctacgccagaaaggccgccaggcaggccagggcaccggtgaagattcctaacattggtaatgtgatgaataaatttgagatccttggggttgtaggtgaaggagcctatggagttgtacttaaatgcagacacaaggaaacacatgaaattgtggcgatcaagaaattcaaggacagtgaagaaaatgaagaagtcaaagaaacgactttacgagagcttaaaatgcttcggactctcaagcaggaaaacattgtggagttgaaggaagcatttcgtcggaggggaaagttgtacttggtgtttgagtatgttgaaaaaaatatgctcgaattgctggaagaaatgccaaatggagttccacctgagaaagtaaaaagctacatctatcagctaatcaaggctattcactggtgccataagaatgatattgtccatcgagatataaaaccagaaaatctcttaatcagccacaatgatgtcctaaaactgtgtgactttggttttgctcgtaatctgtcagaaggcaataatgctaattacacagagtacgttgccaccagatggtatcggtccccagaactcttacttggcgctccctatggaaagtccgtggacatgtggtcggtgggctgtattcttggggagcttagcgatggacagcctttatttcctggagaaagtgaaattgaccaactttttactattcagaaggtgctaggaccacttccatctgagcagatgaagcttttctacagtaatcctcgcttccatgggctccggtttccagctgttaaccatcctcagtccttggaaagaagataccttggaattttgaatagtgttctacttgacctaatgaagaatttactgaagttggacccagctgacagatacttgacagaacagtgtttgaatcaccctacatttcaaacccagagacttctggatcgttctccttcaaggtcagcaaaaagaaaaccttaccatgtggaaagcagcacattgtctaatagaaaccaagccggcaaaagcactgctttgcagtctcaccacagatctaacagcaaggacatccagaacctgagtgtaggcctgccccgggctgacgaaggtctccctgccaatgaaagcttcctaaatggaaaccttgctggagctagtcttagtccactgcacaccaaaacctaccaagcaagcagccagcctgggtctaccagcaaagatctcaccaacaacaacataccacaccttcttagcccaaaagaagccaagtcaaaaacagagtttgattttaatattgacccaaagccttcagaaggcccagggacaaagtacctcaagtcaaacagcagatctcagcagaaccgccactcattcatggaaagctctcaaagcaaagctgggacactgcagcccaatgaaaagcagagtcggcatagctatattgacacaattccccagtcctctaggagtccctcctacaggaccaaggccaaaagccatggggcactgagtgactccaagtctgtgagcaacctttctgaagccagggcccaaattgcggagcccagtaccagtaggtacttcccatctagctgcttagacttgaattctcccaccagcccaacccccaccagacacagtgacacgagaactttgctcagcccttctggaagaaataaccgaaatgagggaacgctggactcacgtcgaaccacaaccagacattctaagacgatggaggaattgaagctgccggagcacatggacagtagccattcccattcactgtctgcacctcacgaatctttttcttatggactgggctacaccagccccttttcttcccagcaacgtcctcataggcattctatgtatgtgacccgtgacaaagtgagagccaagggcttggatggaagcttgagcatagggcaagggatggcagctagagccaacagcctgcaactcttgtcaccccagcctggagaacagctccctccagagatgactgtggcaagatcttcggtcaaagagacctccagagaaggcacctcttccttccatacacgccagaagtctgagggtggagtgtatcatgacccacactctgatgatggcacagcccccaaagaaaatagacacctatacaatgatcctgtgccaaggagagttggtagcttttacagagtgccatctccacgtccagacaattctttccatgaaaataatgtgtcaactagagtttcttctctaccatcagagagcagttctggaaccaaccactcaaaaagacaaccagcattcgatccatggaaaagtcctgaaaatattagtcattcggagcaactcaaggaaaaagagaagcaaggatttttcaggtcaatgaaaaagaaaaagaagaaatctcaaacagtacccaattccgacagccctgatcttctgacgttgcagaaatccattcattctgctagcactccaagcagcagaccaaaggagtggcgccccgagaagatctcagatctgcagacccaaagccagccattaaagtcactgcgcaagttgttacatctctcttcggcctcaaatcacccggcttcctcagatccccgcttccagcccttaacagctcaacaaaccaaaaattccttctcagaaattcggattcaccccctgagccaggcctctggcgggagcagcaacatccggcaggaacccgcaccgaagggcaggccagccctccagctgccaggtcagatggatcctggttggcatgtgtcctctgtgaccaggagtgccacagagggcccttcctactctgaacagctgggtgccaaaagtgggccaaatgggcacccctataacagaacaaatcgctcacgaatgccaaatctgaatgatttaaaagagacagccttgtctagaggatcccgggctgactacaaagaccatgacggtgattataaagatcatgacatcgactacaaggatgacgatgacaagtaggagctcaagctttctttgaaccaaaattagaaaaccaaggcttgaaacgttcaattgaaatggcaattaaacaaattacagcacgtgttgctttgattgatagccaaaaagcagcagttgataaagcaattactgatattgctgaaaaattgtaatttataaataaaaatcaccttttagaggtggtttttttatttataaattattcgtttgatttcgctttcgatagaacaatcaaatcgtttctgagacgttttagcgtttatttcgtttagttatcggcataatcgttaaaacaggcgttatcgtagcgtaaaagcccttgagcgtagcgtgctttgcagcgaagatgttgtctgttagattatgaaagccgatgactgaatgaaataataagcgcagcgtccttctatttcggttggaggaggctcaagggagtttgagggaatgaaattccctcatgggtttgattttaaaaattgcttgcaattttgccgagcggtagcgctggaaaatttttgaaaaaaatttggaatttggaaaaaaatggggggaaaggaagcgaattttgcttccgtactacgaccccccattaagtgccgagtgccaatttttgtgccaaaaacgctctatcccaactggctcaagggtttgaggggtttttcaatcgccaacgaatcgccaacgttttcgccaacgttttttataaatctatatttaagtagctttattgttgtttttatgattacaaagtgatacactaattttataaaattatttgattggagttttttaaatggtgatttcagaatcgaaaaaaagagttatgatttctctgacaaaagagcaagataaaaaattaacagatatggcgaaacaaaaaggtttttcaaaatctgcggttgcggcgttagctatagaagaatatgcaagaaaggaatcagaacaaaaaaaataagcgaaagctcgcgtttttagaaggatacgagttttcgctacttgtttttgataaggtaatatatcatggctattaaaaatactaaagctagaaattttggatttttattatatcctgactcaattcctaatgattggaaagaaaaattagagagtttgggcgtatctatggctgtcagtcctttacacgatatggacgaaaaaaaagataaagatacatggaatagtagtgatgttatacgaaatggaaagcactataaaaaaccacactatcacgttatatatattgcacgaaatcctgtaacaatagaaagcgttaggaacaagattaagcgaaaattggggaatagttcagttgctcatgttgagatacttgattatatcaaaggttcatatgaatatttgactcatgaatcaaaggacgctattgctaagaataaacatatatacgacaaaaaagatattttgaacattaatgattttgatattgaccgctatataacacttgatgaaagccaaaaaagagaattgaagaatttacttttagatatagtggatgactataatttggtaaatacaaaagatttaatggcttttattcgccttaggggagcggagtttggaattttaaatacgaatgatgtaaaagatattgtttcaacaaactctagcgcctttagattatggtttgagggcaattatcagtgtggatatagagcaagttatgcaaaggttcttgatgctgaaacgggggaaataaaatgacaaacaaagaaaaagagttatttgctgaaaatgaggaattaaaaaaagaaattaaggacttaaaagagcgtattgaaagatacagagaaatggaagttgaattaagtacaacaatagatttattgagaggagggattattgaataaataaaagcccccctgacgaaagtcgacggcaatagttacccttattatcaagataagaaagaaaaggatttttcgctacgctcaaatcctttaaaaaaacacaaaagaccacattttttaatgtggtctttattcttcaactaaagcacccattagttcaacaaacgaaaattggataaagtgggatatttttaaaatatatatttatgttacagtaatattgacttttaaaaaaggattgattctaatgaagaaagcagacaagtaagcctcctaaattcactttagataaaaatttaggaggcatatcaaatgaactttaataaaattgatttagacaattggaagagaaaagagatatttaatcattatttgaaccaacaaacgacttttagtataaccacagaaattgatattagtgttttataccgaaacataaaacaagaaggatataaattttaccctgcatttattttcttagtgacaagggtgataaactcaaatacagcttttagaactggttacaatagcgacggagagttaggttattgggataagttagagccactttatacaatttttgatggtgtatctaaaacattctctggtatttggactcctgtaaagaatgacttcaaagagttttatgatttatacctttctgatgtagagaaatataatggttcggggaaattgtttcccaaaacacctatacctgaaaatgctttttctctttctattattccttggacttcatttactgggtttaacttaaatatcaataataatagtaattaccttctacccattattacagcaggaaaattcattaataaaggtaattcaatatatttaccgctatctttacaggtacatcattctgtttgtgatggttatcatgcaggattgtttatgaactctattcaggaattgtcagataggcctaatgactggcttttataatatgagataatgccgactgtactttttacagtcggttttctaatgtcactaacctgccccgttagttgaagaaggtttttatattacagctcca

SEQ ID NO: 23 - protein, 1036 aa, synthetic construct
METDTLLLWVLLLWVPGSTGDAAQPARRARRTKLAAYARKAARQARAPVKIPNIGNVMNKFEILGVVGEGAYGVVLKCRHKETHEIVAIKKFKDSEENEEVKETTLRELKMLRTLKQENIVELKEAFRRRGKLYLVFEYVEKNMLELLEEMPNGVPPEKVKSYIYQLIKAIHWCHKNDIVHRDIKPENLLISHNDVLKLCDFGFARNLSEGNNANYTEYVATRWYRSPELLLGAPYGKSVDMWSVGCILGELSDGQPLFPGESEIDQLFTIQKVLGPLPSEQMKLFYSNPRFHGLRFPAVNHPQSLERRYLGILNSVLLDLMKNLLKLDPADRYLTEQCLNHPTFQTQRLLDRSPSRSAKRKPYHVESSTLSNRNQAGKSTALQSHHRSNSKDIQNLSVGLPRADEGLPANESFLNGNLAGASLSPLHTKTYQASSQPGSTSKDLTNNNIPHLLSPKEAKSKTEFDFNIDPKPSEGPGTKYLKSNSRSQQNRHSFMESSQSKAGTLQPNEKQSRHSYIDTIPQSSRSPSYRTKAKSHGALSDSKSVSNLSEARAQIAEPSTSRYFPSSCLDLNSPTSPTPTRHSDTRTLLSPSGRNNRNEGTLDSRRTTTRHSKTMEELKLPEHMDSSHSHSLSAPHESFSYGLGYTSPFSSQQRPHRHSMYVTRDKVRAKGLDGSLSIGQGMAARANSLQLLSPQPGEQLPPEMTVARSSVKETSREGTSSFHTRQKSEGGVYHDPHSDDGTAPKENRHLYNDPVPRRVGSFYRVPSPRPDNSFHENNVSTRVSSLPSESSSGTNHSKRQPAFDPWKSPENISHSEQLKEKEKQGFFRSMKKKKKKSQTVPNSDSPDLLTLQKSIHSASTPSSRPKEWRPEKISDLQTQSQPLKSLRKLLHLSSASNHPASSDPRFQPLTAQQTKNSFSEIRIHPLSQASGGSSNIRQEPAPKGRPALQLPGQMDPGWHVSSVTRSATEGPSYSEQLGAKSGPNGHPYNRTNRSRMPNLNDLKETALSRGSRADYKDHDGDYKDHDIDYKDDDDK

SEQ ID NO: 24 - DNA, 6350 bp, synthetic construct
  source 1..6350: mol_type = other DNA
agatctagtcttataactatactgacaatagaaacattaacaaatctaaaacagtcttaattctatcttgagaaagtattggtaataatattattgtcgataacgcgagcataataaacggctctgattaaattctgaagtttgttagatacaatgatttcgttcgaaggaactacaaaataaattataaggaggcactcaccatgggtactgcaggcatgcggtaccttatggctaaaaaaaagattatctcagctattttaatgtctacagtgatactttctgctgcagccccgttgtcaggtgtttacgctatggagacagacacactcctgctatgggtactgctgctctgggttccaggttccactggtgacgcggcccagccggccaggcgcgcgcgccgtacgaagcttgcggcctacgccagaaaggccgccaggcaggccagggcaccggtgaagattcctaacattggtaatgtgatgaataaatttgagatccttggggttgtaggtgaaggagcctatggagttgtacttaaatgcagacacaaggaaacacatgaaattgtggcgatcaagaaattcaaggacagtgaagaaaatgaagaagtcaaagaaacgactttacgagagcttaaaatgcttcggactctcaagcaggaaaacattgtggagttgaaggaagcatttcgtcggaggggaaagttgtacttggtgtttgagtatgttgaaaaaaatatgctcgaattgctggaagaaatgccaaatggagttccacctgagaaagtaaaaagctacatctatcagctaatcaaggctattcactggtgccataagaatgatattgtccatcgagatataaaaccagaaaatctcttaatcagccacaatgatgtcctaaaactgtgtgactttggttttgctcgtaatctgtcagaaggcaataatgctaattacacagagtacgttgccaccagatggtatcggtccccagaactcttacttggcgctccctatggaaagtccgtggacatgtggtcggtgggctgtattcttggggagcttagcgatggacagcctttatttcctggagaaagtgaaattgaccaactttttactattcagaaggtgctaggaccacttccatctgagcagatgaagcttttctacagtaatcctcgcttccatgggctccggtttccagctgttaaccatcctcagtccttggaaagaagataccttggaattttgaatagtgttctacttgacctaatgaagaatttactgaagttggacccagctgacagatacttgacagaacagtgtttgaatcaccctacatttcaaacccagagacttctggatcgttctccttcaaggtcagcaaaaagaaaaccttaccatgtggaaagcagcacattgtctaatagaaaccaagccggcaaaagcactgctttgcagtctcaccacagatctaacagcaaggacatccagaacctgagtgtaggcctgccccgggctgacgaaggtctccctgccaatgaaagcttcctaaatggaaaccttgctggagctagtcttagtccactgcacaccaaaacctaccaagcaagcagccagcctgggtctaccagcaaagatctcaccaacaacaacataccacaccttcttagcccaaaagaagccaagtcaaaaacagagtttgattttaatattgacccaaagccttcagaaggcccagggacaaagtacctcaagtcaaacagcagatctcagcagaaccgccactcattcatggaaagctctcaaagcaaagctgggacactgcagcccaatgaaaagcagagtcggcatagctatattgacacaattccccagtcctctaggagtccctcctacaggaccaaggccaaaagccatggggcactgagtgactccaagtctgtgagcaacctttctgaagccagggcccaaattgcggagcccagtaccagtaggtacttcccatctagctgcttagacttgaattctcccaccagcccaacccccaccagacacagtgacacgagaactttgctcagcccttctggaagaaataaccgaaatgagggaacgctggactcacgtcgaaccacaaccagacattctaagacgatggaggaattgaagctgccggagcacatggacagtagccattcccattcactgtctgcacctcacgaatctttttcttatggactgggctacaccagccccttttcttcccagcaacgtcctcataggcattctatgtatgtgacccgtgacaaagtgagagccaagggcttggatggaagcttgagcatagggcaagggatggcagctagagccaacagcctgcaactcttgtcaccccagcctggagaacagctccctccagagatgactgtggcaagatcttcggtcaaagagacctccagagaaggcacctcttccttccatacacgccagaagtctgagggtggagtgtatcatgacccacactctgatgatggcacagcccccaaagaaaatagacacctatacaatgatcctgtgccaaggagagttggtagcttttacagagtgccatctccacgtccagacaattctttccatgaaaataatgtgtcaactagagtttcttctctaccatcagagagcagttctggaaccaaccactcaaaaagacaaccagcattcgatccatggaaaagtcctgaaaatattagtcattcggagcaactcaaggaaaaagagaagcaaggatttttcaggtcaatgaaaaagaaaaagaagaaatctcaaacagtacccaattccgacagccctgatcttctgacgttgcagaaatccattcattctgctagcactccaagcagcagaccaaaggagtggcgccccgagaagatctcagatctgcagacccaaagccagccattaaagtcactgcgcaagttgttacatctctcttcggcctcaaatcacccggcttcctcagatccccgcttccagcccttaacagctcaacaaaccaaaaattccttctcagaaattcggattcaccccctgagccaggcctctggcgggagcagcaacatccggcaggaacccgcaccgaagggcaggccagccctccagctgccaggtcagatggatcctggttggcatgtgtcctctgtgaccaggagtgccacagagggcccttcctactctgaacagctgggtgccaaaagtgggccaaatgggcacccctataacagaacaaatcgctcacgaatgccaaatctgaatgatttaaaagagacagccttgtctagaggatcccgggctgactacaaagaccatgacggtgattataaagatcatgacatcgactacaaggatgacgatgacaagtaggagctcaagctttctttgaaccaaaattagaaaaccaaggcttgaaacgttcaattgaaatggcaattaaacaaattacagcacgtgttgctttgattgatagccaaaaagcagcagttgataaagcaattactgatattgctgaaaaattgtaatttataaataaaaatcaccttttagaggtggtttttttatttataaattattcgtttgatttcgctttcgatagaacaatcaaatcgtttctgagacgttttagcgtttatttcgtttagttatcggcataatcgttaaaacaggcgttatcgtagcgtaaaagcccttgagcgtagcgtgctttgcagcgaagatgttgtctgttagattatgaaagccgatgactgaatgaaataataagcgcagcgtccttctatttcggttggaggaggctcaagggagtttgagggaatgaaattccctcatgggtttgattttaaaaattgcttgcaattttgccgagcggtagcgctggaaaatttttgaaaaaaatttggaatttggaaaaaaatggggggaaaggaagcgaattttgcttccgtactacgaccccccattaagtgccgagtgccaatttttgtgccaaaaacgctctatcccaactggctcaagggtttgaggggtttttcaatcgccaacgaatcgccaacgttttcgccaacgttttttataaatctatatttaagtagctttattgttgtttttatgattacaaagtgatacactaattttataaaattatttgattggagttttttaaatggtgatttcagaatcgaaaaaaagagttatgatttctctgacaaaagagcaagataaaaaattaacagatatggcgaaacaaaaaggtttttcaaaatctgcggttgcggcgttagctatagaagaatatgcaagaaaggaatcagaacaaaaaaaataagcgaaagctcgcgtttttagaaggatacgagttttcgctacttgtttttgataaggtaatatatcatggctattaaaaatactaaagctagaaattttggatttttattatatcctgactcaattcctaatgattggaaagaaaaattagagagtttgggcgtatctatggctgtcagtcctttacacgatatggacgaaaaaaaagataaagatacatggaatagtagtgatgttatacgaaatggaaagcactataaaaaaccacactatcacgttatatatattgcacgaaatcctgtaacaatagaaagcgttaggaacaagattaagcgaaaattggggaatagttcagttgctcatgttgagatacttgattatatcaaaggttcatatgaatatttgactcatgaatcaaaggacgctattgctaagaataaacatatatacgacaaaaaagatattttgaacattaatgattttgatattgaccgctatataacacttgatgaaagccaaaaaagagaattgaagaatttacttttagatatagtggatgactataatttggtaaatacaaaagatttaatggcttttattcgccttaggggagcggagtttggaattttaaatacgaatgatgtaaaagatattgtttcaacaaactctagcgcctttagattatggtttgagggcaattatcagtgtggatatagagcaagttatgcaaaggttcttgatgctgaaacgggggaaataaaatgacaaacaaagaaaaagagttatttgctgaaaatgaggaattaaaaaaagaaattaaggacttaaaagagcgtattgaaagatacagagaaatggaagttgaattaagtacaacaatagatttattgagaggagggattattgaataaataaaagcccccctgacgaaagtcgacggcaatagttacccttattatcaagataagaaagaaaaggatttttcgctacgctcaaatcctttaaaaaaacacaaaagaccacattttttaatgtggtctttattcttcaactaaagcacccattagttcaacaaacgaaaattggataaagtgggatatttttaaaatatatatttatgttacagtaatattgacttttaaaaaaggattgattctaatgaagaaagcagacaagtaagcctcctaaattcactttagataaaaatttaggaggcatatcaaatgaactttaataaaattgatttagacaattggaagagaaaagagatatttaatcattatttgaaccaacaaacgacttttagtataaccacagaaattgatattagtgttttataccgaaacataaaacaagaaggatataaattttaccctgcatttattttcttagtgacaagggtgataaactcaaatacagcttttagaactggttacaatagcgacggagagttaggttattgggataagttagagccactttatacaatttttgatggtgtatctaaaacattctctggtatttggactcctgtaaagaatgacttcaaagagttttatgatttatacctttctgatgtagagaaatataatggttcggggaaattgtttcccaaaacacctatacctgaaaatgctttttctctttctattattccttggacttcatttactgggtttaacttaaatatcaataataatagtaattaccttctacccattattacagcaggaaaattcattaataaaggtaattcaatatatttaccgctatctttacaggtacatcattctgtttgtgatggttatcatgcaggattgtttatgaactctattcaggaattgtcagataggcctaatgactggcttttataatatgagataatgccgactgtactttttacagtcggttttctaatgtcactaacctgccccgttagttgaagaaggtttttatattacagctcca

SEQ ID NO: 25 - protein, 1064 aa, synthetic construct
MAKKKIISAILMSTVILSAAAPLSGVYAMETDTLLLWVLLLWVPGSTGDAAQPARRARRTKLAAYARKAARQARAPVKIPNIGNVMNKFEILGVVGEGAYGVVLKCRHKETHEIVAIKKFKDSEENEEVKETTLRELKMLRTLKQENIVELKEAFRRRGKLYLVFEYVEKNMLELLEEMPNGVPPEKVKSYIYQLIKAIHWCHKNDIVHRDIKPENLLISHNDVLKLCDFGFARNLSEGNNANYTEYVATRWYRSPELLLGAPYGKSVDMWSVGCILGELSDGQPLFPGESEIDQLFTIQKVLGPLPSEQMKLFYSNPRFHGLRFPAVNHPQSLERRYLGILNSVLLDLMKNLLKLDPADRYLTEQCLNHPTFQTQRLLDRSPSRSAKRKPYHVESSTLSNRNQAGKSTALQSHHRSNSKDIQNLSVGLPRADEGLPANESFLNGNLAGASLSPLHTKTYQASSQPGSTSKDLTNNNIPHLLSPKEAKSKTEFDFNIDPKPSEGPGTKYLKSNSRSQQNRHSFMESSQSKAGTLQPNEKQSRHSYIDTIPQSSRSPSYRTKAKSHGALSDSKSVSNLSEARAQIAEPSTSRYFPSSCLDLNSPTSPTPTRHSDTRTLLSPSGRNNRNEGTLDSRRTTTRHSKTMEELKLPEHMDSSHSHSLSAPHESFSYGLGYTSPFSSQQRPHRHSMYVTRDKVRAKGLDGSLSIGQGMAARANSLQLLSPQPGEQLPPEMTVARSSVKETSREGTSSFHTRQKSEGGVYHDPHSDDGTAPKENRHLYNDPVPRRVGSFYRVPSPRPDNSFHENNVSTRVSSLPSESSSGTNHSKRQPAFDPWKSPENISHSEQLKEKEKQGFFRSMKKKKKKSQTVPNSDSPDLLTLQKSIHSASTPSSRPKEWRPEKISDLQTQSQPLKSLRKLLHLSSASNHPASSDPRFQPLTAQQTKNSFSEIRIHPLSQASGGSSNIRQEPAPKGRPALQLPGQMDPGWHVSSVTRSATEGPSYSEQLGAKSGPNGHPYNRTNRSRMPNLNDLKETALSRGSRADYKDHDGDYKDHDIDYKDDDDK

SEQ ID NO: 26 - protein, 11 aa, synthetic construct
YARKAARQARA

SEQ ID NO: 27 - protein, 28 aa, synthetic construct
MAKKKIISAILMSTVILSAAAPLSGVYA

SEQ ID NO: 28 - protein, 461 aa, Lactococcus sp.
MKKKIISAILMSTVILSAAAPLSGVYADTNSDIAKQDATISSAQSAKAQAQAQVDSLQSKVDSLQQKQTSTKAQIAKIESEAKALNAQIATLNESIKERTKTLEAQARSAQVNSSATNYMDAVVNSKSLTDVIQKVTAIATVSSANKQMLEQQEKEQKELSQKSETVKKNYNQFVSLSQSLDSQAQELTSQQAELKVATLNYQATIATAQDKKQALLDEKAAAEKAAQEAAKKQAAYEAQQKEAAQAQAASTAATAKAVEAATSSASASSSQAPQVSTSTDNTTSNASASNSSNSSSNSSSSSSSSSSSSSSSSNSNAGGNTNSGTSTGNTGGTTTGGSGINSSPIGNPYAGGGCTDYVWQYFAAQGIYIRNIMPGNGGQWASNGPAQGVLHVVGAAPGVIASSFSADFVGYANSPYGHVAIVKSVNSDGTITIKEGGYGTTWWGHERTVSASGVTFLMPN

SEQ ID NO: 29 - protein, 1029 aa, synthetic construct
KIPNIGNVMNKFEILGVVGEGAYGVVLKCRHKETHEIVAIKKFKDSEENEEVKETTLRELKMLRTLKQENIVELKEAFRRRGKLYLVFEYVEKNMLELLEEMPNGVPPEKVKSYIYQLIKAIHWCHKNDIVHRDIKPENLLISHNDVLKLCDFGFARNLSEGNNANYTEYVATRWYRSPELLLGAPYGKSVDMWSVGCILGELSDGQPLFPGESEIDQLFTIQKVLGPLPSEQMKLFYSNPRFHGLRFPAVNHPQSLERRYLGILNSVLLDLMKNLLKLDPADRYLTEQCLNHPTFQTQRLLDRSPSRSAKRKPYHVESSTLSNRNQAGKSTALQSHHRSNSKDIQNLSVGLPRADEGLPANESFLNGNLAGASLSPLHTKTYQASSQPGSTSKDLTNNNIPHLLSPKEAKSKTEFDFNIDPKPSEGPGTKYLKSNSRSQQNRHSFMESSQSKAGTLQPNEKQSRHSYIDTIPQSSRSPSYRTKAKSHGALSDSKSVSNLSEARAQIAEPSTSRYFPSSCLDLNSPTSPTPTRHSDTRTLLSPSGRNNRNEGTLDSRRTTTRHSKTMEELKLPEHMDSSHSHSLSAPHESFSYGLGYTSPFSSQQRPHRHSMYVTRDKVRAKGLDGSLSIGQGMAARANSLQLLSPQPGEQLPPEMTVARSSVKETSREGTSSFHTRQKSEGGVYHDPHSDDGTAPKENRHLYNDPVPRRVGSFYRVPSPRPDNSFHENNVSTRVSSLPSESSSGTNHSKRQPAFDPWKSPENISHSEQLKEKEKQGFFRSMKKKKKKSQTVPNSDSPDLLTLQKSIHSASTPSSRPKEWRPEKISDLQTQSQPLKSLRKLLHLSSASNHPASSDPRFQPLTAQQTKNSFSEIRIHPLSQASGGSSNIRQEPAPKGRPALQLPDGGCDGRRQRHHSGPQDRRFMLRTTEQQGEYFCCGDPKKPHTPCVPNRALHRPISSPAPYPVLQVRGTSMCPTLQVRGTDAFSCPTQQSGFSFFVRHVMREALIHRAQVNQAALLTYHENAALTGK

SEQ ID NO: 30 - protein, 959 aa, synthetic construct
KIPNIGNVMNKFEILGVVGEGAYGVVLKCRHKETHEIVAIKKFKDSEENEEVKETTLRELKMLRTLKQENIVELKEAFRRRGKLYLVFEYVEKNMLELLEEMPNGVPPEKVKSYIYQLIKAIHWCHKNDIVHRDIKPENLLISHNDVLKLCDFGFARNLSEGNNANYTEYVATRWYRSPELLLGAPYGKSVDMWSVGCILGELSDGQPLFPGESEIDQLFTIQKVLGPLPSEQMKLFYSNPRFHGLRFPAVNHPQSLERRYLGILNSVLLDLMKNLLKLDPADRYLTEQCLNHPTFQTQRLLDRSPSRSAKRKPYHVESSTLSNRNQAGKSTALQSHHRSNSKDIQNLSVGLPRADEGLPANESFLNGNLAGASLSPLHTKTYQASSQPGSTSKDLTNNNIPHLLSPKEAKSKTEFDFNIDPKPSEGPGTKYLKSNSRSQQNRHSFMESSQSKAGTLQPNEKQSRHSYIDTIPQSSRSPSYRTKAKSHGALSDSKSVSNLSEARAQIAEPSTSRYFPSSCLDLNSPTSPTPTRHSDTRTLLSPSGRNNRNEGTLDSRRTTTRHSKTMEELKLPEHMDSSHSHSLSAPHESFSYGLGYTSPFSSQQRPHRHSMYVTRDKVRAKGLDGSLSIGQGMAARANSLQLLSPQPGEQLPPEMTVARSSVKETSREGTSSFHTRQKSEGGVYHDPHSDDGTAPKENRHLYNDPVPRRVGSFYRVPSPRPDNSFHENNVSTRVSSLPSESSSGTNHSKRQPAFDPWKSPENISHSEQLKEKEKQGFFRSMKKKKKKSQTVPNSDSPDLLTLQKSIHSASTPSSRPKEWRPEKISDLQTQSQPLKSLRKLLHLSSASNHPASSDPRFQPLTAQQTKNSFSEIRIHPLSQASGGSSNIRQEPAPKGRPALQLPGQMDPGWHVSSVTRSATEGPSYSEQLGAKSGPNGHPYNRTNRSRMPNLNDLKETAL